European Patent Application EP 4 464 795 A1, published November 20, 2024. Title: Method of detecting structural variation. Applicant: 株式会社日立製作所. The sequence listing filed with the application follows.

SEQUENCE LISTING (12 sequences)

SEQ ID NO: 1 - DNA, 20 bp, synthetic construct
  misc_feature 1..20: note = synthetic primer
  misc_feature 1: note = labelled with Fluorescein
  source 1..20: mol_type = other DNA
tctctgtcatagggactctg

SEQ ID NO: 2 - DNA, 20 bp, synthetic construct
  misc_feature 1..20: note = synthetic primer
  misc_feature 1: note = labelled with Cy3
  source 1..20: mol_type = other DNA
tctctgtcatagggactctg

SEQ ID NO: 3 - DNA, 20 bp, synthetic construct
  misc_feature 1..20: note = synthetic primer
  misc_feature 1: note = labelled with Fluorescein
  misc_feature 7: note = labelled with Cy3
  source 1..20: mol_type = other DNA
tctctgtcatagggactctg

SEQ ID NO: 4 - DNA, 20 bp, synthetic construct
  misc_feature 1..20: note = synthetic primer
  misc_feature 1: note = labelled with Fluorescein
  misc_feature 7: note = labelled with Cy3
  misc_feature 17: note = labelled with Cy3
  source 1..20: mol_type = other DNA
tctctgtcatagggactctg

SEQ ID NO: 5 - DNA, 20 bp, synthetic construct
  misc_feature 1..20: note = synthetic primer
  source 1..20: mol_type = other DNA
ggatttccttgttggctttc

SEQ ID NO: 6 - DNA, 18 bp, synthetic construct
  misc_feature 1..18: note = synthetic primer
  misc_feature 1: note = labelled with Fluorescein
  misc_feature 11: note = labelled with Cy3
  source 1..18: mol_type = other DNA
cacactgacgtgcctctc

SEQ ID NO: 7 - DNA, 16 bp, synthetic construct
  misc_feature 1..16: note = synthetic primer
  source 1..16: mol_type = other DNA
gctgcgtgatgagctg

SEQ ID NO: 8 - DNA, 19 bp, synthetic construct
  misc_feature 1..19: note = synthetic primer
  source 1..19: mol_type = other DNA
gtgtgctccctggatattc

SEQ ID NO: 9 - DNA, 19 bp, synthetic construct
  misc_feature 1..19: note = synthetic primer
  misc_feature 1: note = labelled with Fluorescein
  misc_feature 15: note = labelled with Cy3
  source 1..19: mol_type = other DNA
gtgtgctccctggatattc

SEQ ID NO: 10 - DNA, 23 bp, synthetic construct
  misc_feature 1..23: note = synthetic primer
  source 1..23: mol_type = other DNA
ctcctgagacctttgataacata

SEQ ID NO: 11 - DNA, 23 bp, synthetic construct
  misc_feature 1..23: note = synthetic primer
  misc_feature 1: note = labelled with Fluorescein
  misc_feature 5: note = labelled with Cy3
  misc_feature 14: note = labelled with Cy3
  source 1..23: mol_type = other DNA
ctcctgagacctttgataacata

SEQ ID NO: 12 - DNA, 20 bp, synthetic construct
  misc_feature 1..20: note = synthetic primer
  misc_feature 1: note = labelled with Fluorescein
  source 1..20: mol_type = other DNA
gctttctcccactgtattga